European Patent Specification EP 3 655 958 B1, published September 16, 2026. Title: GENOMIC SERVICES PLATFORM SUPPORTING MULTIPLE APPLICATION PROVIDERS. Applicant: Lu, James Chou, Jim Lee, William Williams, Chris Warren, James Jiang, Ruomu Helix OpCo, LLC. The sequence listing filed with the application follows.

SEQUENCE LISTING (1 sequence)

SEQ ID NO: 1 - DNA, 18 bp, Artificial Sequence
  A synthetic oligonucleotide sequence
attcgtactaacgttggc